European Patent Application EP 4 786 586 A1, published August 5, 2026. Title: 利用RNA剪接调节剂调控基因表达的核酸分子. Applicant: 北京大学. The sequence listing filed with the application follows.

SEQUENCE LISTING (46 sequences)

SEQ ID NO: 1 - DNA, 84 bp, Mus musculus domesticus
  source 1..84: mol_type = genomic DNA
gttaaaggattacatattaaaaatattgtatagactctttaaggccaaagaagtgtgctcatttctcccgattaaaagttatga

SEQ ID NO: 2 - DNA, 39 bp, Mus musculus domesticus
  source 1..39: mol_type = genomic DNA
actgaccaacagcgtgaagacattacatccagtgcacag

SEQ ID NO: 3 - DNA, 500 bp, synthetic construct
  source 1..500: mol_type = other DNA
gtaattgaattcttgttggattactgtctctaaggcctgggagttttataattgtttctttatgtgtaataataaccgtactagtcattgtgatacttatttgggaagtaagcctttaaagaggttattaaaaagatttactgattcccacaccggaagttgctcttctagccgtgaaagaaggacggcgtggtcttcagtttgctatgtccactaacaatatgtccgacccacgaaggcccaccaaagttatacttgtggcacatataaacctttggaatcaagggacctgatactggattattaaatatttaagagaatttatatttaataaacttgatacttcagtgagaaaggacaaatcatcagtagaatggttttgagatagctgatgattctattaaaagtagatatgtgtgtgggttaaatgacttaagcatacatcaaaagactgagaaaggctcttaacattaaaagatgggcctttttttttcttttag

SEQ ID NO: 4 - DNA, 140 bp, synthetic construct
  source 1..140: mol_type = other DNA
gtaattgaattcttgttggattactgtctctaaggcctgggagttagtagatatgtgtgtgggttaaatgacttaagcatacatcaaaagactgagaaaggctcttaacattaaaagatgggcctttttttttcttttag

SEQ ID NO: 5 - DNA, 110 bp, synthetic construct
  source 1..110: mol_type = other DNA
gtaattgaattcttgttggattactgtctctaaggcctgggagttagcatacatcaaaagactgagaaaggctcttaacattaaaagatgggcctttttttttcttttag

SEQ ID NO: 6 - DNA, 569 bp, synthetic construct
  source 1..569: mol_type = other DNA
gtaagaattgggtattttgccttttgggggtgggagatttgaaacagggtttctccttacagctctggctttcctggagcagtgaattgagcctggctcctctgtaggagtaacgagttgctttaaccactgacatctttccaccaccaccaccaccccttatgaatagactaaatttatttaaagattgatattttctagcttaattatttggaaagcaaataagcacacagaaaagcctcctccccaaaaaaatataaataaaaaagtctatcaggacatagtatatgtcccttctgattaatcattggtggtgaaacaacccattcagggtgtctcttccatcacagtggatttttttcatattgttacatggagaagttaacttagtaagaattgatgtgcttctgtgccagtgagatagctctgcaggtaaaagggagactgacccccaacttgtactctggccgtggcagtcatgtgcacacaagtaaactgaataaatataaagagcagattttagagtgttttggctttaaattaattctatattctaactctatttgcag

SEQ ID NO: 7 - DNA, 209 bp, synthetic construct
  source 1..209: mol_type = other DNA
gtaagaattgggtattttgccttttgggggtgggagatttgaaacagggtttccagtgagatagctctgcaggtaaaagggagactgacccccaacttgtactctggccgtggcagtcatgtgcacacaagtaaactgaataaatataaagagcagattttagagtgttttggctttaaattaattctatattctaactctatttgcag

SEQ ID NO: 8 - DNA, 129 bp, synthetic construct
  source 1..129: mol_type = other DNA
gtaagaattgggtattttgccttttgggggtgggagtgagatagctctgcaggtaaaagggagactgacccccaacttgtactctggccgtggctttaaattaattctatattctaactctatttgcag

SEQ ID NO: 9 - DNA, 42 bp, Mus musculus domesticus
  source 1..42: mol_type = genomic DNA
tttgcattgagactccttgcattccgtcagatacacaaagtt

SEQ ID NO: 10 - DNA, 1234 bp, synthetic construct
  source 1..1234: mol_type = other DNA
actgaccaacagcgtgaagacattacatccagtgcacaggtaattgaattcttgttggattactgtctctaaggcctgggagttttataattgtttctttatgtgtaataataaccgtactagtcattgtgatacttatttgggaagtaagcctttaaagaggttattaaaaagatttactgattcccacaccggaagttgctcttctagccgtgaaagaaggacggcgtggtcttcagtttgctatgtccactaacaatatgtccgacccacgaaggcccaccaaagttatacttgtggcacatataaacctttggaatcaagggacctgatactggattattaaatatttaagagaatttatatttaataaacttgatacttcagtgagaaaggacaaatcatcagtagaatggttttgagatagctgatgattctattaaaagtagatatgtgtgtgggttaaatgacttaagcatacatcaaaagactgagaaaggctcttaacattaaaagatgggcctttttttttcttttaggttaaaggattacatattaaaaatattgtatagactctttaaggccaaagaagtgtgctcatttctcccgattaaaagttatgagtaagaattgggtattttgccttttgggggtgggagatttgaaacagggtttctccttacagctctggctttcctggagcagtgaattgagcctggctcctctgtaggagtaacgagttgctttaaccactgacatctttccaccaccaccaccaccccttatgaatagactaaatttatttaaagattgatattttctagcttaattatttggaaagcaaataagcacacagaaaagcctcctccccaaaaaaatataaataaaaaagtctatcaggacatagtatatgtcccttctgattaatcattggtggtgaaacaacccattcagggtgtctcttccatcacagtggatttttttcatattgttacatggagaagttaacttagtaagaattgatgtgcttctgtgccagtgagatagctctgcaggtaaaagggagactgacccccaacttgtactctggccgtggcagtcatgtgcacacaagtaaactgaataaatataaagagcagattttagagtgttttggctttaaattaattctatattctaactctatttgcagtttgcattgagactccttgcattccgtcagatacacaaagtt

SEQ ID NO: 11 - DNA, 514 bp, synthetic construct
  source 1..514: mol_type = other DNA
actgaccaacagcgtgaagacattacatccagtgcacaggtaattgaattcttgttggattactgtctctaaggcctgggagttagtagatatgtgtgtgggttaaatgacttaagcatacatcaaaagactgagaaaggctcttaacattaaaagatgggcctttttttttcttttaggttaaaggattacatattaaaaatattgtatagactctttaaggccaaagaagtgtgctcatttctcccgattaaaagttatgagtaagaattgggtattttgccttttgggggtgggagatttgaaacagggtttccagtgagatagctctgcaggtaaaagggagactgacccccaacttgtactctggccgtggcagtcatgtgcacacaagtaaactgaataaatataaagagcagattttagagtgttttggctttaaattaattctatattctaactctatttgcagtttgcattgagactccttgcattccgtcagatacacaaagtt

SEQ ID NO: 12 - DNA, 404 bp, synthetic construct
  source 1..404: mol_type = other DNA
actgaccaacagcgtgaagacattacatccagtgcacaggtaattgaattcttgttggattactgtctctaaggcctgggagttagcatacatcaaaagactgagaaaggctcttaacattaaaagatgggcctttttttttcttttaggttaaaggattacatattaaaaatattgtatagactctttaaggccaaagaagtgtgctcatttctcccgattaaaagttatgagtaagaattgggtattttgccttttgggggtgggagtgagatagctctgcaggtaaaagggagactgacccccaacttgtactctggccgtggctttaaattaattctatattctaactctatttgcagtttgcattgagactccttgcattccgtcagatacacaaagtt

SEQ ID NO: 13 - DNA, 57 bp, synthetic construct
  source 1..57: mol_type = other DNA
gctactaacttcagcctactaaaacaggctggagacgttgaggagaaccctggacct

SEQ ID NO: 14 - RNA, 81 nt, synthetic construct
  source 1..81: mol_type = other RNA
actgaccaacagcgtgaagacattacatccagtgcacagtttgcattgagactccttgcattccgtcagatacacaaagtt

SEQ ID NO: 15 - RNA, 165 nt, synthetic construct
  source 1..165: mol_type = other RNA
actgaccaacagcgtgaagacattacatccagtgcacaggttaaaggattacatattaaaaatattgtatagactctttaaggccaaagaagtgtgctcatttctcccgattaaaagttatgatttgcattgagactccttgcattccgtcagatacacaaagtt

SEQ ID NO: 16 - DNA, 23 bp, synthetic construct
  source 1..23: mol_type = other DNA
ttatgatttgcattgagactcct

SEQ ID NO: 17 - DNA, 25 bp, synthetic construct
  source 1..25: mol_type = other DNA
gaagtgtgctcatttctcccgatta

SEQ ID NO: 18 - DNA, 24 bp, synthetic construct
  source 1..24: mol_type = other DNA
cgtgaagacattacatccagtgca

SEQ ID NO: 19 - DNA, 15 bp, synthetic construct
  source 1..15: mol_type = other DNA
taaggcctgggagtt

SEQ ID NO: 20 - DNA, 26 bp, synthetic construct
  source 1..26: mol_type = other DNA
agcatacatcaaaagactgagaaagg

SEQ ID NO: 21 - DNA, 60 bp, synthetic construct
  source 1..60: mol_type = other DNA
agtgagatagctctgcaggtaaaagggagactgacccccaacttgtactctggccgtggc

SEQ ID NO: 22 - DNA, 410 bp, synthetic construct
  source 1..410: mol_type = other DNA
gtaattgaattcttgttggattactgtctctaaggcctgggagttatttactgattcccacaccggaagttgctcttctagccgtgaaagaaggacggcgtggtcttcagtttgctatgtccactaacaatatgtccgacccacgaaggcccaccaaagttatacttgtggcacatataaacctttggaatcaagggacctgatactggattattaaatatttaagagaatttatatttaataaacttgatacttcagtgagaaaggacaaatcatcagtagaatggttttgagatagctgatgattctattaaaagtagatatgtgtgtgggttaaatgacttaagcatacatcaaaagactgagaaaggctcttaacattaaaagatgggcctttttttttcttttag

SEQ ID NO: 23 - DNA, 410 bp, synthetic construct
  source 1..410: mol_type = other DNA
gtaattgaattcttgttggattactgtctctaaggcctgggagttttataattgtttctttatgtgtaataataaccgtactagtcattgtgatacttatttgggaagtaagcctttaaagaggttattaaaaagccgacccacgaaggcccaccaaagttatacttgtggcacatataaacctttggaatcaagggacctgatactggattattaaatatttaagagaatttatatttaataaacttgatacttcagtgagaaaggacaaatcatcagtagaatggttttgagatagctgatgattctattaaaagtagatatgtgtgtgggttaaatgacttaagcatacatcaaaagactgagaaaggctcttaacattaaaagatgggcctttttttttcttttag

SEQ ID NO: 24 - DNA, 410 bp, synthetic construct
  source 1..410: mol_type = other DNA
gtaattgaattcttgttggattactgtctctaaggcctgggagttttataattgtttctttatgtgtaataataaccgtactagtcattgtgatacttatttgggaagtaagcctttaaagaggttattaaaaagatttactgattcccacaccggaagttgctcttctagccgtgaaagaaggacggcgtggtcttcagtttgctatgtccactaacaatatgtgagaatttatatttaataaacttgatacttcagtgagaaaggacaaatcatcagtagaatggttttgagatagctgatgattctattaaaagtagatatgtgtgtgggttaaatgacttaagcatacatcaaaagactgagaaaggctcttaacattaaaagatgggcctttttttttcttttag

SEQ ID NO: 25 - DNA, 410 bp, synthetic construct
  source 1..410: mol_type = other DNA
gtaattgaattcttgttggattactgtctctaaggcctgggagttttataattgtttctttatgtgtaataataaccgtactagtcattgtgatacttatttgggaagtaagcctttaaagaggttattaaaaagatttactgattcccacaccggaagttgctcttctagccgtgaaagaaggacggcgtggtcttcagtttgctatgtccactaacaatatgtccgacccacgaaggcccaccaaagttatacttgtggcacatataaacctttggaatcaagggacctgatactggattattaaatatttaaagtagatatgtgtgtgggttaaatgacttaagcatacatcaaaagactgagaaaggctcttaacattaaaagatgggcctttttttttcttttag

SEQ ID NO: 26 - DNA, 479 bp, synthetic construct
  source 1..479: mol_type = other DNA
gtaagaattgggtattttgccttttgggggtgggagatttgaaacagggtttctccttacagctctggctttcctggagcagtgaattgagcctggctcctctgtaggagtaacgagttgctttaaccactgacatctttccaaaaagcctcctccccaaaaaaatataaataaaaaagtctatcaggacatagtatatgtcccttctgattaatcattggtggtgaaacaacccattcagggtgtctcttccatcacagtggatttttttcatattgttacatggagaagttaacttagtaagaattgatgtgcttctgtgccagtgagatagctctgcaggtaaaagggagactgacccccaacttgtactctggccgtggcagtcatgtgcacacaagtaaactgaataaatataaagagcagattttagagtgttttggctttaaattaattctatattctaactctatttgcag

SEQ ID NO: 27 - DNA, 479 bp, synthetic construct; identical to SEQ ID NO: 26
  source 1..479: mol_type = other DNA

SEQ ID NO: 28 - DNA, 479 bp, synthetic construct
  source 1..479: mol_type = other DNA
gtaagaattgggtattttgccttttgggggtgggagatttgaaacagggtttctccttacagctctggctttcctggagcagtgaattgagcctggctcctctgtaggagtaacgagttgctttaaccactgacatctttccaccaccaccaccaccccttatgaatagactaaatttatttaaagattgatattttctagcttaattatttggaaagcaaataagcacacagccattcagggtgtctcttccatcacagtggatttttttcatattgttacatggagaagttaacttagtaagaattgatgtgcttctgtgccagtgagatagctctgcaggtaaaagggagactgacccccaacttgtactctggccgtggcagtcatgtgcacacaagtaaactgaataaatataaagagcagattttagagtgttttggctttaaattaattctatattctaactctatttgcag

SEQ ID NO: 29 - DNA, 479 bp, synthetic construct
  source 1..479: mol_type = other DNA
gtaagaattgggtattttgccttttgggggtgggagatttgaaacagggtttctccttacagctctggctttcctggagcagtgaattgagcctggctcctctgtaggagtaacgagttgctttaaccactgacatctttccaccaccaccaccaccccttatgaatagactaaatttatttaaagattgatattttctagcttaattatttggaaagcaaataagcacacagaaaagcctcctccccaaaaaaatataaataaaaaagtctatcaggacatagtatatgtcccttctgattaatcattggtggtgaaacaaccagtgagatagctctgcaggtaaaagggagactgacccccaacttgtactctggccgtggcagtcatgtgcacacaagtaaactgaataaatataaagagcagattttagagtgttttggctttaaattaattctatattctaactctatttgcag

SEQ ID NO: 30 - DNA, 189 bp, synthetic construct
  source 1..189: mol_type = other DNA
gtaagaattgggtattttgccttttgggggtgggagtgagatagctctgcaggtaaaagggagactgacccccaacttgtactctggccgtggcagtcatgtgcacacaagtaaactgaataaatataaagagcagattttagagtgttttggctttaaattaattctatattctaactctatttgcag

SEQ ID NO: 31 - DNA, 179 bp, synthetic construct
  source 1..179: mol_type = other DNA
gtaagaattgggtattttgccttttgggggtgggagatttgaaacagggtttccagtgagatagctctgcaggtaaaagggagactgacccccaacttgtactctggccgtggctataaagagcagattttagagtgttttggctttaaattaattctatattctaactctatttgcag

SEQ ID NO: 32 - DNA, 179 bp, synthetic construct
  source 1..179: mol_type = other DNA
gtaagaattgggtattttgccttttgggggtgggagatttgaaacagggtttccagtgagatagctctgcaggtaaaagggagactgacccccaacttgtactctggccgtggcagtcatgtgcacacaagtaaactgaataaatttaaattaattctatattctaactctatttgcag

SEQ ID NO: 33 - DNA, 1201 bp, synthetic construct
  source 1..1201: mol_type = other DNA
gacgtcacaaggagctggtacttattggtaggtatcagggaggaagtctgccaaatcggctggtggggaggtggctctgttatactgactccttagtgattaacaattaatcctgatgtagtctgctaagacagaagtagagtttttagtactttgattttctatatcaatttttcttctattttctttctgttcttgaaaacccttgagagagtgcttgtatagtctgtcccctggagatctgtgtttattacacagtgctgactgtacaagcgaccttgtgatttttatccccttctgaggttgttacacaaagccacattctgccctaaatggttcttaacctaaaaaagcctcatagcacaggagcggtaagtagcatgctgctatatcccaggctgagaaagccccgggcttagaattctttgtagtaatgaggggctctagtggaagcagatgaaggggcgtgccattcagaacatgcggaatgagccctgctctcctaactgagcttctgattgctaggtggacagtgagctgcgtttctgtttctctgatgtacgcttggggaagtggtgcctatagtcaagagtaagtttctaagttaaaaccttgaaattctatgtttaaaatagaggttacatttatagtgtttacttgacttgggagatagtgtgggttagagtgactgtcactaagtgacacaaaaatgaacagagttggtacctctgggaaagaggtttgcacctctattgtataggacttgcacttaagctttgttatgtgttagcgtgttctttttaaaaagtgtggacagcctctctctctctctctctctctctctctctctctctctctctctttctctctctttctctctcatatgttgggtataagggtgtgtgggtgtgggtgcgcgtgtgcacattttatataaaatgtttgtttgtttattgtgaggcaaggtctttctccttaactctgattgttctgattgtcgctattcacagtttcacccccctttgcccctgttcctcagtgctgagtgctcagtttttaaccctttatttgcctttttgtatacagcttggatttatatatttaattttctgagtgttttatttctgttttctcctaggtatttaccaccagagtgttttgtggttgggaaagagccaccaaagatctcaaataaagtcga

SEQ ID NO: 34 - DNA, 452 bp, synthetic construct
  source 1..452: mol_type = other DNA
gtgggtggtctcccagaagaacaagttgccacgtgagcagaaatcggctgggactgactgggcccctggtctctgactctgtaacaaatgatgggtaatagaggaatgggtgcggatggatggtagctgtaactttggcctcaaccgatctcctgaccctctctcagttcctgcaatgctatccatggcagcatgcctttggtgggacctgtgaaccatcagccctgacccttgaccctcatacccacctcctgccaccatggattctgtcttgttactgagctggccaccctgtgaacacagtcaagagtaggcacaggggcatcctcatccctagccgtggtttatgggctgtgttagaattgtagctgaatgtgagaggatgcctctgactgacccctcctggtatcagggtgcttgatcggacctctgtgggcatcggcttgaaagga

SEQ ID NO: 35 - DNA, 1044 bp, synthetic construct
  source 1..1044: mol_type = other DNA
atttgagactgctcctggtgtgatacatccaggtgcctaattgccccggatatttttacagatttttatgaattgaaatatctgtggatatgtggatttttctgtctttctgctttttttttctttctacctttttctttaatcttctgtgtccacttttacctccccaaaatgtattcatttagtaaatatttggcatttacattgactgagctttgtgctgtgggaatgtaaaccctaagttttgtagaacatttcattttactgttgctagtttccttagtcataactgaacttccagtataggaaagcatcaagcacaagtatatatatcaagttaccagtgtacagaaagaaaattcttgcacaaagaacctaggttaggtaactatttagtccattctaactccaggtttatattaagtgctaactcatttggacttccatttattgcagatgaggcagatttcagggagaagagagccaccatggggaagaactgtaagagtaagaggctattatttgtgacttgtatttccctgtagcaaataatttctattagcaaaaaaattttttttgtttgttttttaaagattgatttattttatgtatatgagtacactgtcactctattcagacacatcagaagaaggcatcaaatcccattacagatggttgtgggccaccatgtgggtgctgggaattgaactcaggacctctggaagagcagtcagtgctcttaactgctgagccatctcttttgtgtatctcatccattcctgttacagctctgtaatccaattggctatgaaatcataatcttattaaaaactatactttggtgtttctaaagagtttttccctatctctgaagtcaacaacttctttctgtttgctaaattctaataatcatactattgcttgtcaaaatgttaatgcagtattgttgtctgaacatgttttatgacactaaatttattttacctttttttcccctcctaggtgcatggaggactgcaacagaagagtggggaactgaagtag

SEQ ID NO: 36 - DNA, 982 bp, synthetic construct
  source 1..982: mol_type = other DNA
actcaagcacagcaggagaaagcggaggtcccagtgtcagctgacaagtgagttccagcttcccacatgtgaaattatgaacatgcaccaccttttatatttagtaatgctataaatataagtccttagacatagtaaggagttacctgtggttattgatttagcttacaaaaatcaagggccatattttttttttttatttaatttagcagagatccagatggtcccgagtagccttgcacacactgaccactgaaagcatccttcaaaacacaaccaaagtcaggcagcgggggctcacccctttaatcccagcactaaggaggctgaagcaggtagatctcccaagtttgaggccagcctggttacagagtgagtcccaggacagccagggctacatggagaaaccctgtctcaagaaatacaaccaagaagtgcacgctgtggctcattatgtaaatggaggctctcacaggtataattttaagatctgatttagcatattgatactttttaccccatgggctttagacgtcatttgcttacagtcactgcatcggtaaaggagctctcacttggaatatggtttatttcagtgaaactcctctagctggatgtgatcataacattgtggtcattgaggcagaagtatcatgaaaagggggacagcctgggctatgtagtgatattgaggttagcctgatctatataaactttcagaaaacccaggcatagtggcttatacttataccagtactcaagcaactgccaccatggagacaagaattgccgcagatttgaggccatcctacgctatagagtaagttccagtccacctgggctataatgtaagaccttgtctgaaagagaaaatcaaaagcatcctagtctttgagaatggagtaaaaggtaatttttctatgaaatcttttccttttgctttagagtgtcctcgcatctacagcacggtttcagcttgatc

SEQ ID NO: 37 - DNA, 1034 bp, synthetic construct
  source 1..1034: mol_type = other DNA
tgaaattgacaaatcaccgcactggtaagcttcagattccgacttagtttgccatagttttcaaacctcataggttcctagatatctaaacattgtatgttaatccttcaaagattctgagcagggattacagaccctcgaagtctttgaccaattgccagaggcttttacaactgtcattgtatccttgtcatatttcactaaagacaaaaaatttcacccctaatattgttttcagttaagtctcttctttgtttccactggcactgtgctcctgtgacattggggatatgtttctgctactctttaggacaccttttgatcactgtatgactatagtgtctttaaccattacatctataattaaaacaagaaaaaaaaagatgaaaggcacatatgtactattctacaattcatgaagtatggtttcctagaagtcacccatatgcctctgcttaaatctctttacaatcacagatgggagtcttcagcctgccctactgccactgcaaaggaaaagcaatgagtaagaactctgggtttgttgatggtgtcaatggctaatgccacatcatgctttacatctgaagtcctgtctctctgcctgctctgattatcattatctttcaaatgtaaatacctggtatctctcatgcattaaccttgcacatcggatgtcagtaccatttgtgacacttacctgactttccagcctcagtaggcaaagggaaatctaagagtttgcttacagctgctttgattgtcaactgactgaatttgaagcatttagacatgtattagttacttactcattgctgtgggggaatggcaaaaaaaataccttaggacaagttgtttcccccccccccttggggcttgtagttaaagggtacagctcatcgtggaggaaacatgatgtcagaaaaagattgacccagctgctcacactatatccacagtcaggatacagactgaccgaatgctgctactcatgctctttctcctttctattcagcttcaggaccccagcccat

SEQ ID NO: 38 - DNA, 21 bp, synthetic construct
  source 1..21: mol_type = other DNA
aagctcatttcctggtatgac

SEQ ID NO: 39 - DNA, 21 bp, synthetic construct
  source 1..21: mol_type = other DNA
cttactccttggaggccatgt

SEQ ID NO: 40 - DNA, 19 bp, synthetic construct
  source 1..19: mol_type = other DNA
caacagggtggtggacctc

SEQ ID NO: 41 - DNA, 21 bp, synthetic construct
  source 1..21: mol_type = other DNA
tgaacttgtggccgtttacgt

SEQ ID NO: 42 - DNA, 1470 bp, synthetic construct
  source 1..1470: mol_type = other DNA
gatcccgggcagcagccgccgcctcaaccggccccccagggccaagggcagccgccttcgcagcccccgcaggggcagggcccgccgtccggacccgggcaaccggcacccgcggcgacccaggcggcgccgcaggcaccccccgccgggcatcagatcgtgcacgtccgcggggactcggagaccgacctggaggcgctcttcaacgccgtcatgaaccccaagacggccaacgtgccccagaccgtgcccatgaggctccggaagctgcccgactccttcttcaagccgccggagcccaaatcccactcccgacaggccagtactgatgcaggcactgcaggagccctgactccacagcatgttcgagctcatgcctctccagcttctctgcagttgggagctgtttctcctgggacactgacccccactggagtagtctctggcccagcagctacacccacagctcagcatcttcgacagtcttcttttgagatacctgatgatgtacctctgccagcaggttgggagatggcaaagacatcttctggtcagagatacttcttaaatcacatcgatcagacaacaacatggcaggaccccaggaaggccatgctgtcccagatgaacgtcacagcccccaccagtccaccagtgcagcagaatatgatgaactcggcttcaggtcctcttcctgatggatgggaacaagccatgactcaggatggagaaatttactatataaaccataagaacaagaccacctcttggctagacccaaggcttgaccctcgttttgccatgaaccagagaatcagtcagagtgctccagtgaaacagccaccacccctggctccccagagcccacagggaggcgtcatgggtggcagcaactccaaccagcagcaacagatgcgactgcagcaactgcagatggagaaggagaggctgcggctgaaacagcaagaactgcttcggcaggagttagccctgcgtagccagttaccaacactggagcaggatggtgggactcaaaatccagtgtcttctcccgggatgtctcaggaattgagaacaatgacgaccaatagctcagatcctttccttaacagtggcacctatcactctcgagatgagagtacagacagtggactaagcatgagcagctacagtgtccctcgaaccccagatgacttcctgaacagtgtggatgagatggatacaggtgatactatcaaccaaagcaccctgccctcacagcagaaccgtttcccagactaccttgaagccattcctgggacaaatgtggaccttggaacactggaaggagatggaatgaacatagaaggagaggagctgatgccaagtctgcaggaagctttgagttctgacatccttaatgacatggagtctgttttggctgccaccaagctagataaagaaagctttcttacatggttgtacctctag

SEQ ID NO: 43 - DNA, 1470 bp, synthetic construct
  source 1..1470: mol_type = other DNA
gatcccgggcagcagccgccgcctcaaccggccccccagggccaagggcagccgccttcgcagcccccgcaggggcagggcccgccgtccggacccgggcaaccggcacccgcggcgacccaggcggcgccgcaggcaccccccgccgggcatcagatcgtgcacgtccgcggggacgcggagaccgacctggaggcgctcttcaacgccgtcatgaaccccaagacggccaacgtgccccagaccgtgcccatgaggctccggaagctgcccgactccttcttcaagccgccggagcccaaatcccactcccgacaggccgctactgatgcaggcactgcaggagccctgactccacagcatgttcgagctcatgccgctccagctgctctgcagttgggagctgtttctcctgggacactgacccccactggagtagtctctggcccagcagctacacccacagctcagcatcttcgacaggctgcttttgagatacctgatgatgtacctctgccagcaggttgggagatggcaaagacatcttctggtcagagatacttcttaaatcacatcgatcagacaacaacatggcaggaccccaggaaggccatgctgtcccagatgaacgtcacagcccccaccagtccaccagtgcagcagaatatgatgaactcggcttcaggtcctcttcctgatggatgggaacaagccatgactcaggatggagaaatttactatataaaccataagaacaagaccacctcttggctagacccaaggcttgaccctcgttttgccatgaaccagagaatcagtcagagtgctccagtgaaacagccaccacccctggctccccagagcccacagggaggcgtcatgggtggcagcaactccaaccagcagcaacagatgcgactgcagcaactgcagatggagaaggagaggctgcggctgaaacagcaagaactgcttcggcaggagttagccctgcgtagccagttaccaacactggagcaggatggtgggactcaaaatccagtgtcttctcccgggatgtctcaggaattgagaacaatgacgaccaatagctcagatcctttccttaacagtggcacctatcactctcgagatgaggctacagacagtggactaagcatgagcagctacagtgtccctcgaaccccagatgacttcctgaacagtgtggatgagatggatacaggtgatactatcaaccaaagcaccctgccctcacagcagaaccgtttcccagactaccttgaagccattcctgggacaaatgtggaccttggaacactggaaggagatggaatgaacatagaaggagaggagctgatgccaagtctgcaggaagctttgagttctgacatccttaatgacatggagtctgttttggctgccaccaagctagataaagaaagctttcttacatggttgtacctctag

SEQ ID NO: 44 - RNA, 21 nt, synthetic construct
  source 1..21: mol_type = other RNA
gtatgaaaatccctactggac

SEQ ID NO: 45 - DNA, 24 bp, synthetic construct
  source 1..24: mol_type = other DNA
aagctgaccctgaagttcatctgc

SEQ ID NO: 46 - DNA, 24 bp, synthetic construct
  source 1..24: mol_type = other DNA
cttgtagttgccgtcgtccttgaa